European Patent Application EP 4 364 755 A1, published May 8, 2024. Title: Composition for controlling growth of Clostridium difficile comprising a monoclonal antibody. Applicant: The University of Tokyo. The sequence listing filed with the application follows.

SEQUENCE LISTING (82 sequences)

SEQ ID NO: 1 - protein, 5 aa, Artificial Sequence
  Comment
SYGIS

SEQ ID NO: 2 - protein, 16 aa, Artificial Sequence
  Comment
EIYPRSGNTYYNEKFK

SEQ ID NO: 3 - protein, 8 aa, Artificial Sequence
  Comment
FCARLASS

SEQ ID NO: 4 - protein, 11 aa, Artificial Sequence
  Comment
KASQDINSYLS

SEQ ID NO: 5 - protein, 7 aa, Artificial Sequence
  Comment
RANRLVD

SEQ ID NO: 6 - protein, 9 aa, Artificial Sequence
  Comment
LQYDEFPLT

SEQ ID NO: 7 - protein, 144 aa, Artificial Sequence
  Comment
MEWIWIFLFILSGTAGVQSQVQLQQSGAELARPGASVKLSCKASGYTFTSYGISWVKQRTGQGLEWIGEIYPRSGNTYYNEKFKGKATLTADKSSSTAYMELRSLTSEDSAVYFCARLASSYYGSSYDWYFDVWGTGTTVTVSS

SEQ ID NO: 8 - protein, 127 aa, Artificial Sequence
  Comment
MRTPAQFLGILLLWFPGIKCDIKMTQSPSSMYASLGERVTITCKASQDINSYLSWFQQKPGKSPKTLIYRANRLVDGVPSRFSGSGSGQDYSLTISSLEYEDMGIYYCLQYDEFPLTFGAGTKLELK

SEQ ID NO: 9 - protein, 488 aa, Artificial Sequence
  Comment
MEWIWIFLFILSGTAGVQSQVQLQQSGAELARPGASVKLSCKASGYTFTSYGISWVKQRTGQGLEWIGEIYPRSGNTYYNEKFKGKATLTADKSSSTAYMELRSLTSEDSAVYFCARLASSYYGSSYDWYFDVWGTGTTVTVSSESARNPTIYPLTLPRALSSDPVIIGCLIHDYFPSGTMNVTWGKSGKDITTVNFPPALASGGGYTMSSQLTLPAVECPEGESVKCSVQHDSNAVQELDVKCSGPPPPCPPCPPSCHPSLSLQRPALEDLLLGSDASLTCTLNGLRNPEGAVFTWEPSTGKDAVQKKAVQNSCGCYSVSSVLPGCAERWNSGASFKCTVTHPESDTLTGTIAKITVNTFPPQVHLLPPPSEELALNELVSLTCLVRAFNPKEVLVRWLHGNEELSPESYLVFEPLKEPGEGATTYLVTSVLRVSAELWKQGDQYSCMVGHEALPMNFTQKTIDRLSGKPTNVSVSVIMSEGDGICY

SEQ ID NO: 10 - protein, 234 aa, Artificial Sequence
  Comment
MRTPAQFLGILLLWFPGIKCDIKMTQSPSSMYASLGERVTITCKASQDINSYLSWFQQKPGKSPKTLIYRANRLVDGVPSRFSGSGSGQDYSLTISSLEYEDMGIYYCLQYDEFPLTFGAGTKLELKRADAAPTVSIFPPSSEQLTSGGASVVCFLNNFYPKDINVKWKIDGSERQNGVLNSWTDQDSKDSTYSMSSTLTLTKDEYERHNSYTCEATHKTSTSPIVKSFNRNEC

SEQ ID NO: 11 - protein, 5 aa, Artificial Sequence
  Comment
TFGMG

SEQ ID NO: 12 - protein, 16 aa, Artificial Sequence
  Comment
LAHIWWDDDKYYNPAL

SEQ ID NO: 13 - protein, 8 aa, Artificial Sequence
  Comment
YYCARIAG

SEQ ID NO: 14 - protein, 11 aa, Artificial Sequence
  Comment
SASSSVSYMHW

SEQ ID NO: 15 - protein, 8 aa, Artificial Sequence
  Comment
STSNLASG

SEQ ID NO: 16 - protein, 9 aa, Artificial Sequence
  Comment
QRSSYPYTF

SEQ ID NO: 17 - protein, 135 aa, Artificial Sequence
  Comment
MGRLTSSFLLLIVPAYVLSQVTLKESGPGILQPSQTLSLTCSFSGFSLSTFGMGVGWIRQPSGKGLEWLAHIWWDDDKYYNPALKSRLTISKDTSKNQVFLKIANVDTADTATYYCARIAGFDYWGQGTTLTVSS

SEQ ID NO: 18 - protein, 128 aa, Artificial Sequence
  Comment
MHFQVQIFSFLLISASVIMSRGQIVLTQSPAIMSASPGEKVTITCSASSSVSYMHWFQQKPGTSPKLWIYSTSNLASGVPARFSGSGSGTSYSLTISRMEAEDAATYYCQQRSSYPYTFGGGTKLEIK

SEQ ID NO: 19 - protein, 479 aa, Artificial Sequence
  Comment
MGRLTSSFLLLIVPAYVLSQVTLKESGPGILQPSQTLSLTCSFSGFSLSTFGMGVGWIRQPSGKGLEWLAHIWWDDDKYYNPALKSRLTISKDTSKNQVFLKIANVDTADTATYYCARIAGFDYWGQGTTLTVSSESARNPTIYPLTLPRALSSDPVIIGCLIHDYFPSGTMNVTWGKSGKDITTVNFPPALASGGGYTMSSQLTLPAVECPEGESVKCSVQHDSNAVQELDVKCSGPPPPCPPCPPSCHPSLSLQRPALEDLLLGSDASLTCTLNGLRNPEGAVFTWEPSTGKDAVQKKAVQNSCGCYSVSSVLPGCAERWNSGASFKCTVTHPESDTLTGTIAKITVNTFPPQVHLLPPPSEELALNELVSLTCLVRAFNPKEVLVRWLHGNEELSPESYLVFEPLKEPGEGATTYLVTSVLRVSAELWKQGDQYSCMVGHEALPMNFTQKTIDRLSGKPTNVSVSVIMSEGDGICY

SEQ ID NO: 20 - protein, 235 aa, Artificial Sequence
  Comment
MHFQVQIFSFLLISASVIMSRGQIVLTQSPAIMSASPGEKVTITCSASSSVSYMHWFQQKPGTSPKLWIYSTSNLASGVPARFSGSGSGTSYSLTISRMEAEDAATYYCQQRSSYPYTFGGGTKLEIKRADAAPTVSIFPPSSEQLTSGGASVVCFLNNFYPKDINVKWKIDGSERQNGVLNSWTDQDSKDSTYSMSSTLTLTKDEYERHNSYTCEATHKTSTSPIVKSFNRNEC

SEQ ID NO: 21 - protein, 5 aa, Artificial Sequence
  Comment
SYNIH

SEQ ID NO: 22 - protein, 16 aa, Artificial Sequence
  Comment
AIYSGNGATSHNQKFK

SEQ ID NO: 23 - protein, 8 aa, Artificial Sequence
  Comment
FCTRVGLR

SEQ ID NO: 24 - protein, 11 aa, Artificial Sequence
  Comment
KASQSVGTSVA

SEQ ID NO: 25 - protein, 7 aa, Artificial Sequence
  Comment
SASYRYS

SEQ ID NO: 26 - protein, 9 aa, Artificial Sequence
  Comment
QQYNNYPYT

SEQ ID NO: 27 - protein, 137 aa, Artificial Sequence
  Comment
MGFSRIFLFLLSVTTGVHSQAYLQQSGAELVRPGASVRMSCKASDYTFTSYNIHWVKQTPRQGLEWIGAIYSGNGATSHNQKFKGRATLTVDKSSSTAYMQLSSLTSEDSAVYFCTRVGLRSPFDFWGQGTTLTVSS

SEQ ID NO: 28 - protein, 127 aa, Artificial Sequence
  Comment
MESQTQVFVYMLLWLSGVDGDIVMTQSLKFMSTSGGDRVSVTCKASQSVGTSVAWYQQKPGQSPKPLIYSASYRYSGVPDRFTGSGSGTDFSLTISNVQSEDLAEYFCQQYNNYPYTFGGGTKLEIK

SEQ ID NO: 29 - protein, 481 aa, Artificial Sequence
  Comment
MGFSRIFLFLLSVTTGVHSQAYLQQSGAELVRPGASVRMSCKASDYTFTSYNIHWVKQTPRQGLEWIGAIYSGNGATSHNQKFKGRATLTVDKSSSTAYMQLSSLTSEDSAVYFCTRVGLRSPFDFWGQGTTLTVSSESARNPTIYPLTLPRALSSDPVIIGCLIHDYFPSGTMNVTWGKSGKDITTVNFPPALASGGGYTMSSQLTLPAVECPEGESVKCSVQHDSNAVQELDVKCSGPPPPCPPCPPSCHPSLSLQRPALEDLLLGSDASLTCTLNGLRNPEGAVFTWEPSTGKDAVQKKAVQNSCGCYSVSSVLPGCAERWNSGASFKCTVTHPESDTLTGTIAKITVNTFPPQVHLLPPPSEELALNELVSLTCLVRAFNPKEVLVRWLHGNEELSPESYLVFEPLKEPGEGATTYLVTSVLRVSAELWKQGDQYSCMVGHEALPMNFTQKTIDRLSGKPTNVSVSVIMSEGDGICY

SEQ ID NO: 30 - protein, 234 aa, Artificial Sequence
  Comment
MESQTQVFVYMLLWLSGVDGDIVMTQSLKFMSTSGGDRVSVTCKASQSVGTSVAWYQQKPGQSPKPLIYSASYRYSGVPDRFTGSGSGTDFSLTISNVQSEDLAEYFCQQYNNYPYTFGGGTKLEIKRADAAPTVSIFPPSSEQLTSGGASVVCFLNNFYPKDINVKWKIDGSERQNGVLNSWTDQDSKDSTYSMSSTLTLTKDEYERHNSYTCEATHKTSTSPIVKSFNRNEC

SEQ ID NO: 31 - protein, 5 aa, Artificial Sequence
  Comment
DYYIH

SEQ ID NO: 32 - protein, 16 aa, Artificial Sequence
  Comment
RIDPENDETTYAPKFQ

SEQ ID NO: 33 - protein, 8 aa, Artificial Sequence
  Comment
YCARSTVL

SEQ ID NO: 34 - protein, 11 aa, Artificial Sequence
  Comment
RASQSIVHTNG

SEQ ID NO: 35 - protein, 7 aa, Artificial Sequence
  Comment
KLLIYKV

SEQ ID NO: 36 - protein, 9 aa, Artificial Sequence
  Comment
GVYYCFQGS

SEQ ID NO: 37 - protein, 134 aa, Artificial Sequence
  Comment
MKCSWIIFFLMAVVTGVNSEVQLQQSGSELVKSGASVKLSCTVSGFNFTDYYIHWVRQRTEQGLEWIGRIDPENDETTYAPKFQGKATMTADTSSNTAYLQLTSLTSEDTAVYYCARSTVLDYWGHGTTLTVSS

SEQ ID NO: 38 - protein, 131 aa, Artificial Sequence
  Comment
MKLPVRLLVLMFWIPGFSSDVLMTQTPLSLPVSLGDQASISCRASQSIVHTNGNTYLEWYLQKPGQSPKLLIYKVSNRFSGVPDRFSGSGSGTDFILKISRVEAEDLGVYYCFQGSHVPPTFGGGTKLEVK

SEQ ID NO: 39 - protein, 478 aa, Artificial Sequence
  Comment
MKCSWIIFFLMAVVTGVNSEVQLQQSGSELVKSGASVKLSCTVSGFNFTDYYIHWVRQRTEQGLEWIGRIDPENDETTYAPKFQGKATMTADTSSNTAYLQLTSLTSEDTAVYYCARSTVLDYWGHGTTLTVSSESARNPTIYPLTLPRALSSDPVIIGCLIHDYFPSGTMNVTWGKSGKDITTVNFPPALASGGGYTMSSQLTLPAVECPEGESVKCSVQHDSNAVQELDVKCSGPPPPCPPCPPSCHPSLSLQRPALEDLLLGSDASLTCTLNGLRNPEGAVFTWEPSTGKDAVQKKAVQNSCGCYSVSSVLPGCAERWNSGASFKCTVTHPESDTLTGTIAKITVNTFPPQVHLLPPPSEELALNELVSLTCLVRAFNPKEVLVRWLHGNEELSPESYLVFEPLKEPGEGATTYLVTSVLRVSAELWKQGDQYSCMVGHEALPMNFTQKTIDRLSGKPTNVSVSVIMSEGDGICY

SEQ ID NO: 40 - protein, 238 aa, Artificial Sequence
  Comment
MKLPVRLLVLMFWIPGFSSDVLMTQTPLSLPVSLGDQASISCRASQSIVHTNGNTYLEWYLQKPGQSPKLLIYKVSNRFSGVPDRFSGSGSGTDFILKISRVEAEDLGVYYCFQGSHVPPTFGGGTKLEVKRADAAPTVSIFPPSSEQLTSGGASVVCFLNNFYPKDINVKWKIDGSERQNGVLNSWTDQDSKDSTYSMSSTLTLTKDEYERHNSYTCEATHKTSTSPIVKSFNRNEC

SEQ ID NO: 41 - protein, 5 aa, Artificial Sequence
  Comment
NYYIH

SEQ ID NO: 42 - protein, 16 aa, Artificial Sequence
  Comment
RIDPENNETTYAPKFQ

SEQ ID NO: 43 - protein, 16 aa, Artificial Sequence
  Comment
RIDPENDQTTYAPKFQ

SEQ ID NO: 44 - protein, 16 aa, Artificial Sequence
  Comment
RIDPENNQTTYAPKFQ

SEQ ID NO: 45 - protein, 134 aa, Artificial Sequence
  Comment
MKCSWIIFFLMAVVTGVNSEVQLQQSGSELVKSGASVKLSCTVSGFNFTNYYIHWVRQRTEQGLEWIGRIDPENDETTYAPKFQGKATMTADTSSNTAYLQLTSLTSEDTAVYYCARSTVLDYWGHGTTLTVSS

SEQ ID NO: 46 - protein, 134 aa, Artificial Sequence
  Comment
MKCSWIIFFLMAVVTGVNSEVQLQQSGSELVKSGASVKLSCTVSGFNFTDYYIHWVRQRTEQGLEWIGRIDPENNETTYAPKFQGKATMTADTSSNTAYLQLTSLTSEDTAVYYCARSTVLDYWGHGTTLTVSS

SEQ ID NO: 47 - protein, 134 aa, Artificial Sequence
  Comment
MKCSWIIFFLMAVVTGVNSEVQLQQSGSELVKSGASVKLSCTVSGFNFTDYYIHWVRQRTEQGLEWIGRIDPENDQTTYAPKFQGKATMTADTSSNTAYLQLTSLTSEDTAVYYCARSTVLDYWGHGTTLTVSS

SEQ ID NO: 48 - protein, 134 aa, Artificial Sequence
  Comment
MKCSWIIFFLMAVVTGVNSEVQLQQSGSELVKSGASVKLSCTVSGFNFTNYYIHWVRQRTEQGLEWIGRIDPENNETTYAPKFQGKATMTADTSSNTAYLQLTSLTSEDTAVYYCARSTVLDYWGHGTTLTVSS

SEQ ID NO: 49 - protein, 134 aa, Artificial Sequence
  Comment
MKCSWIIFFLMAVVTGVNSEVQLQQSGSELVKSGASVKLSCTVSGFNFTNYYIHWVRQRTEQGLEWIGRIDPENDQTTYAPKFQGKATMTADTSSNTAYLQLTSLTSEDTAVYYCARSTVLDYWGHGTTLTVSS

SEQ ID NO: 50 - protein, 134 aa, Artificial Sequence
  Comment
MKCSWIIFFLMAVVTGVNSEVQLQQSGSELVKSGASVKLSCTVSGFNFTDYYIHWVRQRTEQGLEWIGRIDPENNQTTYAPKFQGKATMTADTSSNTAYLQLTSLTSEDTAVYYCARSTVLDYWGHGTTLTVSS

SEQ ID NO: 51 - protein, 134 aa, Artificial Sequence
  Comment
MKCSWIIFFLMAVVTGVNSEVQLQQSGSELVKSGASVKLSCTVSGFNFTNYYIHWVRQRTEQGLEWIGRIDPENNQTTYAPKFQGKATMTADTSSNTAYLQLTSLTSEDTAVYYCARSTVLDYWGHGTTLTVSS

SEQ ID NO: 52 - protein, 11 aa, Artificial Sequence
  Comment
RSSQSIVHTNG

SEQ ID NO: 53 - protein, 13 aa, Artificial Sequence
  Comment
SPASLSVSLGDRA

SEQ ID NO: 54 - protein, 13 aa, Artificial Sequence
  Comment
SPASLSVSLGDRV

SEQ ID NO: 55 - protein, 13 aa, Artificial Sequence
  Comment
SPASMSVSLGDRA

SEQ ID NO: 56 - protein, 13 aa, Artificial Sequence
  Comment
TPLSLPVSLGDQA

SEQ ID NO: 57 - protein, 131 aa, Artificial Sequence
  Comment
MKLPVRLLVLMFWIPGFSSDVLMTQSPASLSVSLGDRATISCRASQSIVHTNGNTYLEWYLQKPGQSPKLLIYKVSNRFSGVPDRFSGSGSGTDFILKISRVEAEDLGVYYCFQGSHVPPTFGGGTKLEVK

SEQ ID NO: 58 - protein, 131 aa, Artificial Sequence
  Comment
MKLPVRLLVLMFWIPGFSSDVLMTQSPASLSVSLGDRVTISCRASQSIVHTNGNTYLEWYLQKPGQSPKLLIYKVSNRFSGVPDRFSGSGSGTDFILKISRVEAEDLGVYYCFQGSHVPPTFGGGTKLEVK

SEQ ID NO: 59 - protein, 131 aa, Artificial Sequence
  Comment
MKLPVRLLVLMFWIPGFSSDVLMTQSPASLSVSLGDRVTISCRSSQSIVHTNGNTYLEWYLQKPGQSPKLLIYKVSNRFSGVPDRFSGSGSGTDFILKISRVEAEDLGVYYCFQGSHVPPTFGGGTKLEVK

SEQ ID NO: 60 - protein, 131 aa, Artificial Sequence
  Comment
MKLPVRLLVLMFWIPGFSSDVLMTQSPASMSVSLGDRATISCRSSQSIVHTNGNTYLEWYLQKPGQSPKLLIYKVSNRFSGVPDRFSGSGSGTDFILKISRVEAEDLGVYYCFQGSHVPPTFGGGTKLEVK

SEQ ID NO: 61 - protein, 131 aa, Artificial Sequence
  Comment
MKLPVRLLVLMFWIPGFSSDVLMTQSPASLSVSLGDRATISCRSSQSIVHTNGNTYLEWYLQKPGQSPKLLIYKVSNRFSGVPDRFSGSGSGTDFILKISRVEAEDLGVYYCFQGSHVPPTFGGGTKLEVK

SEQ ID NO: 62 - protein, 5 aa, Artificial Sequence
  Comment
  misc_feature (1)..(1): Xaa can be any naturally occurring amino acid
XYYIH

SEQ ID NO: 63 - protein, 16 aa, Artificial Sequence
  Comment
  misc_feature (7)..(8): Xaa can be any naturally occurring amino acid
RIDPENXXTTYAPKFQ

SEQ ID NO: 64 - protein, 11 aa, Artificial Sequence
  Comment
  misc_feature (2)..(2): Xaa can be any naturally occurring amino acid
RXSQSIVHTNG

SEQ ID NO: 65 - DNA, 1467 bp, Artificial Sequence
  Comment
atggaatggatctggatctttctcttcatcctgtcaggaactgcaggtgtccaatcccaggttcagctgcagcagtctggagctgagctggcgaggcctggggcttcagtgaagctgtcctgcaaggcttctggctacaccttcacaagctatggtataagctgggtgaagcagagaactggacagggccttgagtggattggagagatttatcctagaagtggtaatacttactacaatgagaagttcaagggcaaggccacactgactgcagacaaatcctccagcacagcgtacatggagctccgcagcctgacatctgaggactctgcggtctatttctgtgcaagattggcatcgagctactacggtagtagctacgactggtacttcgatgtctggggcacagggaccacggtcaccgtctcctcagagtctgcgagaaatcccaccatctacccactgacactcccacgagctctgtcaagtgacccagtgataatcggctgcctgattcacgattacttcccttccggcacgatgaatgtgacctggggaaagagtgggaaggatataaccaccgtaaacttcccacctgccctggcctctgggggagggtacaccatgagcagccagttgaccctgccagctgtcgagtgcccagaaggagaatccgtgaaatgttccgtgcaacatgactctaacgccgtccaagaattggatgtgaagtgctctggtcctcctcctccttgtcctccttgtcctccttcctgccatcccagcctgtcactgcagcggccagctcttgaggacctgctcctgggttcagatgccagcctcacatgtactctgaatggcctgagaaatcctgagggagctgtcttcacctgggagccctccactgggaaggatgcagtgcagaagaaagctgtgcagaattcctgcggctgctacagtgtgtccagcgtcctgcctggctgtgctgagcgctggaacagtggcgcatcattcaagtgcacagttacccatcctgagtctgacaccttaactggcacaattgccaaaatcacagtgaacaccttcccaccccaggtccacctgctaccgccgccgtcggaggagctggccctgaatgagctcgtgtccctgacatgcctggtgcgagctttcaaccctaaagaagtgctggtgcgatggctgcatggaaatgaggagctgtccccagaaagctacctagtgtttgagcccctaaaggagccaggcgagggagccaccacctacctggtgacaagcgtgttgcgtgtatcagctgaactctggaaacagggtgaccagtactcctgcatggtgggccacgaggccttgcccatgaacttcacccagaagaccatcgaccgtctgtcgggtaaacccaccaatgtcagcgtgtctgtgatcatgtcagagggagatggcatctgctactga

SEQ ID NO: 66 - DNA, 705 bp, Artificial Sequence
  Comment
atgaggacccctgctcagtttcttggaatcttgttgctctggtttccaggtatcaaatgtgacatcaagatgacccagtctccatcttccatgtatgcatctctaggagagagagtcactatcacttgcaaggcgagtcaggacattaatagctatttaagctggttccagcagaaaccagggaaatctcctaagaccctgatctatcgtgcaaacagattggtagatggggtcccatcaaggttcagtggcagtggatctgggcaagattattctctcaccatcagcagcctggagtatgaagatatgggaatttattattgtctacagtatgatgagtttccgctcacgttcggtgctgggaccaagctggagctgaaacgggctgatgctgcaccaactgtatccatcttcccaccatccagtgagcagttaacatctggaggtgcctcagtcgtgtgcttcttgaacaacttctaccccaaagacatcaatgtcaagtggaagattgatggcagtgaacgacaaaatggcgtcctgaacagttggactgatcaggacagcaaagacagcacctacagcatgagcagcaccctcacgttgaccaaggacgagtatgaacgacataacagctatacctgtgaggccactcacaagacatcaacttcacccattgtcaagagcttcaacaggaatgagtgttga

SEQ ID NO: 67 - DNA, 1440 bp, Artificial Sequence
  Comment
atgggcaggcttacttcttcattcctgttactgattgtccctgcatatgtcctgtcccaggttactctgaaagagtctggccctgggatattgcagccctcccagaccctcagtctgacttgttctttctctgggttttcactgagcacttttggtatgggtgtaggctggattcgtcagccttcagggaagggtctggagtggctggcacacatttggtgggatgatgataagtactataacccagccctgaagagtcggctcacaatctccaaggatacctccaaaaaccaggtattcctcaagatcgccaatgtggacactgcagatactgccacatactactgtgctcgaatagctgggtttgactactggggccaaggcaccactctcacagtctcctcagagtctgcgagaaatcccaccatctacccactgacactcccacgagctctgtcaagtgacccagtgataatcggctgcctgattcacgattacttcccttccggcacgatgaatgtgacctggggaaagagtgggaaggatataaccaccgtaaacttcccacctgccctggcctctgggggagggtacaccatgagcagccagttgaccctgccagctgtcgagtgcccagaaggagaatccgtgaaatgttccgtgcaacatgactctaacgccgtccaagaattggatgtgaagtgctctggtcctcctcctccttgtcctccttgtcctccttcctgccatcccagcctgtcactgcagcggccagctcttgaggacctgctcctgggttcagatgccagcctcacatgtactctgaatggcctgagaaatcctgagggagctgtcttcacctgggagccctccactgggaaggatgcagtgcagaagaaagctgtgcagaattcctgcggctgctacagtgtgtccagcgtcctgcctggctgtgctgagcgctggaacagtggcgcatcattcaagtgcacagttacccatcctgagtctgacaccttaactggcacaattgccaaaatcacagtgaacaccttcccaccccaggtccacctgctaccgccgccgtcggaggagctggccctgaatgagctcgtgtccctgacatgcctggtgcgagctttcaaccctaaagaagtgctggtgcgatggctgcatggaaatgaggagctgtccccagaaagctacctagtgtttgagcccctaaaggagccaggcgagggagccaccacctacctggtgacaagcgtgttgcgtgtatcagctgaactctggaaacagggtgaccagtactcctgcatggtgggccacgaggccttgcccatgaacttcacccagaagaccatcgaccgtctgtcgggtaaacccaccaatgtcagcgtgtctgtgatcatgtcagagggagatggcatctgctactga

SEQ ID NO: 68 - DNA, 708 bp, Artificial Sequence
  Comment
atgcattttcaagtgcagattttcagcttcctgctaatcagtgcctcagtcataatgtccagaggacaaattgttctcacccagtctccagcaatcatgtctgcatctccaggggagaaggtcaccataacctgcagtgccagctcaagtgtaagttacatgcactggttccagcagaagccaggcacttctcccaaactctggatttatagcacatccaacctggcttctggagtccctgctcgcttcagtggcagtggatctgggacctcttactctctcacaatcagccgaatggaggctgaagatgctgccacttattactgccagcaaaggagtagttacccgtacacgttcggaggggggaccaagctggaaataaaacgggctgatgctgcaccaactgtatccatcttcccaccatccagtgagcagttaacatctggaggtgcctcagtcgtgtgcttcttgaacaacttctaccccaaagacatcaatgtcaagtggaagattgatggcagtgaacgacaaaatggcgtcctgaacagttggactgatcaggacagcaaagacagcacctacagcatgagcagcaccctcacgttgaccaaggacgagtatgaacgacataacagctatacctgtgaggccactcacaagacatcaacttcacccattgtcaagagcttcaacaggaatgagtgttga

SEQ ID NO: 69 - DNA, 1446 bp, Artificial Sequence
  Comment
atgggattcagcaggatctttctcttcctcctgtcagtaactacaggtgtccactcccaggcttatctacagcagtctggggctgagctggtgaggcctggggcctcagtgaggatgtcctgcaaggcttctgactacacatttaccagttacaatatccactgggtaaagcagacacctagacagggcctggaatggattggagctatttattcaggaaatggtgctacttcccacaatcagaagttcaagggcagggccacactgactgtagacaaatcctccagcacagcctacatgcaactcagcagcctgacatctgaagactctgcggtctatttctgtacaagagtgggactccggtccccttttgacttctggggccaaggcaccactctcacagtctcctcagagtctgcgagaaatcccaccatctacccactgacactcccacgagctctgtcaagtgacccagtgataatcggctgcctgattcacgattacttcccttccggcacgatgaatgtgacctggggaaagagtgggaaggatataaccaccgtaaacttcccacctgccctggcctctgggggagggtacaccatgagcagccagttgaccctgccagctgtcgagtgcccagaaggagaatccgtgaaatgttccgtgcaacatgactctaacgccgtccaagaattggatgtgaagtgctctggtcctcctcctccttgtcctccttgtcctccttcctgccatcccagcctgtcactgcagcggccagctcttgaggacctgctcctgggttcagatgccagcctcacatgtactctgaatggcctgagaaatcctgagggagctgtcttcacctgggagccctccactgggaaggatgcagtgcagaagaaagctgtgcagaattcctgcggctgctacagtgtgtccagcgtcctgcctggctgtgctgagcgctggaacagtggcgcatcattcaagtgcacagttacccatcctgagtctgacaccttaactggcacaattgccaaaatcacagtgaacaccttcccaccccaggtccacctgctaccgccgccgtcggaggagctggccctgaatgagctcgtgtccctgacatgcctggtgcgagctttcaaccctaaagaagtgctggtgcgatggctgcatggaaatgaggagctgtccccagaaagctacctagtgtttgagcccctaaaggagccaggcgagggagccaccacctacctggtgacaagcgtgttgcgtgtatcagctgaactctggaaacagggtgaccagtactcctgcatggtgggccacgaggccttgcccatgaacttcacccagaagaccatcgaccgtctgtcgggtaaacccaccaatgtcagcgtgtctgtgatcatgtcagagggagatggcatctgctactga

SEQ ID NO: 70 - DNA, 705 bp, Artificial Sequence
  Comment
atggagtcacagactcaggtctttgtatacatgttgctgtggttgtctggtgttgatggagacattgtgatgacccagtctctaaaattcatgtccacatcgggaggagacagggtcagcgtcacctgcaaggccagtcagagtgtgggtacaagtgtagcctggtatcagcagaaaccaggacaatctcctaaaccactgatttattcggcatcttatcggtacagtggagtccctgatcgcttcacaggcagtggatctgggacagatttcagtctcaccatcagcaatgtgcagtctgaagacttggcagaatatttctgtcagcaatataacaactatccgtacacgttcggaggggggaccaagctggagataaaacgggctgatgctgcaccaactgtatccatcttcccaccatccagtgagcagttaacatctggaggtgcctcagtcgtgtgcttcttgaacaacttctaccccaaagacatcaatgtcaagtggaagattgatggcagtgaacgacaaaatggcgtcctgaacagttggactgatcaggacagcaaagacagcacctacagcatgagcagcaccctcacgttgaccaaggacgagtatgaacgacataacagctatacctgtgaggccactcacaagacatcaacttcacccattgtcaagagcttcaacaggaatgagtgttga

SEQ ID NO: 71 - DNA, 1437 bp, Artificial Sequence
  Comment
atgaaatgcagctggatcatcttcttcctgatggcagtggttacaggggtcaattcagaggttcagctgcagcagtctgggtcagagcttgtgaagtctggggcctcagtcaagttgtcctgcacagtttctgggttcaactttacagactactatatacactgggtgaggcagaggactgaacagggcctggaatggattggaaggattgatcctgagaatgatgaaactacatatgccccgaaattccagggcaaggccactatgacagcagacacatcttccaacacagcctacctgcagctcaccagcctgacatctgaagacactgccgtctattactgtgctagatctacggtccttgactactggggccacggcaccactctcacagtctcctcagagtctgcgagaaatcccaccatctacccactgacactcccacgagctctgtcaagtgacccagtgataatcggctgcctgattcacgattacttcccttccggcacgatgaatgtgacctggggaaagagtgggaaggatataaccaccgtaaacttcccacctgccctggcctctgggggagggtacaccatgagcagccagttgaccctgccagctgtcgagtgcccagaaggagaatccgtgaaatgttccgtgcaacatgactctaacgccgtccaagaattggatgtgaagtgctctggtcctcctcctccttgtcctccttgtcctccttcctgccatcccagcctgtcactgcagcggccagctcttgaggacctgctcctgggttcagatgccagcctcacatgtactctgaatggcctgagaaatcctgagggagctgtcttcacctgggagccctccactgggaaggatgcagtgcagaagaaagctgtgcagaattcctgcggctgctacagtgtgtccagcgtcctgcctggctgtgctgagcgctggaacagtggcgcatcattcaagtgcacagttacccatcctgagtctgacaccttaactggcacaattgccaaaatcacagtgaacaccttcccaccccaggtccacctgctaccgccgccgtcggaggagctggccctgaatgagctcgtgtccctgacatgcctggtgcgagctttcaaccctaaagaagtgctggtgcgatggctgcatggaaatgaggagctgtccccagaaagctacctagtgtttgagcccctaaaggagccaggcgagggagccaccacctacctggtgacaagcgtgttgcgtgtatcagctgaactctggaaacagggtgaccagtactcctgcatggtgggccacgaggccttgcccatgaacttcacccagaagaccatcgaccgtctgtcgggtaaacccaccaatgtcagcgtgtctgtgatcatgtcagagggagatggcatctgctactga

SEQ ID NO: 72 - DNA, 717 bp, Artificial Sequence
  Comment
atgaagttgcctgttaggctgttggtgctgatgttctggattcctggattcagcagtgatgttttgatgacccaaactccactctccctgcctgtcagtcttggagatcaagcctccatctcttgtagagctagtcagagcattgtacacactaatgggaacacctatttagaatggtacctgcagaaaccaggccagtctccaaagctcctgatctacaaagtttccaaccgattttctggggtcccagacaggttcagtggcagtggatctgggacagatttcatactcaagatcagcagagtggaggctgaggatctgggagtttattactgctttcaaggttcacatgttcctccgacgttcggtggaggcaccaagctggaagtcaaacgggctgatgctgcaccaactgtatccatcttcccaccatccagtgagcagttaacatctggaggtgcctcagtcgtgtgcttcttgaacaacttctaccccaaagacatcaatgtcaagtggaagattgatggcagtgaacgacaaaatggcgtcctgaacagttggactgatcaggacagcaaagacagcacctacagcatgagcagcaccctcacgttgaccaaggacgagtatgaacgacataacagctatacctgtgaggccactcacaagacatcaacttcacccattgtcaagagcttcaacaggaatgagtgttag

SEQ ID NO: 73 - DNA, 1374 bp, Artificial Sequence
  Comment
atgaaatgcagctggatcatcttcttcctgatggcagtggttacaggggtcaattcagaggttcagctgcagcagtctgggtcagagcttgtgaagtctggggcctcagtcaagttgtcctgcacagtttctgggttcaactttacagactactatatacactgggtgaggcagaggactgaacagggcctggaatggattggaaggattgatcctgagaatgatgaaactacatatgccccgaaattccagggcaaggccactatgacagcagacacatcttccaacacagcctacctgcagctcaccagcctgacatctgaagacactgccgtctattactgtgctagatctacggtccttgactactggggccacggcaccactctcacagtctcctcaaaaacgacacccccatctgtctatccactggcccctggatctgctgcccaaactaactccatggtgaccctgggatgcctggtcaagggctatttccctgagccagtgacagtgacctggaactctggatccctgtccagcggtgtgcacaccttcccagctgtcctgcagtctgacctctacactctgagcagctcagtgactgtcccctccagcacctggcccagcgagaccgtcacctgcaacgttgcccacccggccagcagcaccaaggtggacaagaaaattgtgcccagggattgtggttgtaagccttgcatatgtacagtcccagaagtatcatctgtcttcatcttccccccaaagcccaaggatgtgctcaccattactctgactcctaaggtcacgtgtgttgtggtagacatcagcaaggatgatcccgaggtccagttcagctggtttgtagatgatgtggaggtgcacacagctcagacgcaaccccgggaggagcagttcaacagcactttccgctcagtcagtgaacttcccatcatgcaccaggactggctcaatggcaaggagttcaaatgcagggtcaacagtgcagctttccctgcccccatcgagaaaaccatctccaaaaccaaaggcagaccgaaggctccacaggtgtacaccattccacctcccaaggagcagatggccaaggataaagtcagtctgacctgcatgataacagacttcttccctgaagacattactgtggagtggcagtggaatgggcagccagcggagaactacaagaacactcagcccatcatggacacagatggctcttacttcgtctacagcaagctcaatgtgcagaagagcaactgggaggcaggaaatactttcacctgctctgtgttacatgagggcctgcacaaccaccatactgagaagagcctctcccactctcctggtaaataa

SEQ ID NO: 74 - DNA, 1407 bp, Artificial Sequence
  Comment
atgaaatgcagctggatcatcttcttcctgatggcagtggttacaggggtcaattcagaggttcagctgcagcagtctgggtcagagcttgtgaagtctggggcctcagtcaagttgtcctgcacagtttctgggttcaactttacagactactatatacactgggtgaggcagaggactgaacagggcctggaatggattggaaggattgatcctgagaatgatgaaactacatatgccccgaaattccagggcaaggccactatgacagcagacacatcttccaacacagcctacctgcagctcaccagcctgacatctgaagacactgccgtctattactgtgctagatctacggtccttgactactggggccacggcaccactctcacagtctcctcagcatccccgactagttccaccaagggcccatcggtcttccccctggcaccctcctccaagagcacctctgggggcacagcggccctgggctgcctggtcaaggactacttccccgaaccggtgacggtgtcgtggaactcaggcgccctgaccagcggcgtgcacaccttcccggctgtcctacagtcctcaggactctactccctcagcagcgtggtgaccgtgccctccagcagcttgggcacccagacctacatctgcaacgtgaatcacaagcccagcaacaccaaggtggacaagaaagttgagcccaaatcttgtgacaaaactcacacatgcccaccgtgcccagcacctgaactcctggggggaccgtcagtcttcctcttccccccaaaacccaaggacaccctcatgatctcccggacccctgaggtcacatgcgtggtggtggacgtgagccacgaagaccctgaggtcaagttcaactggtacgtggacggcgtggaggtgcataatgccaagacaaagccgcgggaggagcagtacaacagcacgtaccgtgtggtcagcgtcctcaccgtcctgcaccaggactggctgaatggcaaggagtacaagtgcaaggtctccaacaaagccctcccagcccctatcgagaaaaccatctccaaagccaaagggcagccccgagaaccacaggtgtacaccctgcccccatcccgggatgagctgaccaagaaccaggtcagcctgacctgcctggtcaaaggcttctatcccagcgacatcgccgtggagtgggagagcaatgggcagccggagaacaactacaagaccacgcctcccgtgctggactccgacggctccttcttcctctacagcaagctcaccgtggacaagagcaggtggcagcaggggaacgtcttctcatgctccgtgatgcatgagggtctgcacaaccactacacgcagaagagcctctccctgtctccgggtaaatga

SEQ ID NO: 75 - DNA, 723 bp, Artificial Sequence
  Comment
atggacatgaagttgcctgttaggctgttggtgctgatgttctggattcctggattcagcagtgatgttttgatgacccaaactccactctccctgcctgtcagtcttggagatcaagcctccatctcttgtagagctagtcagagcattgtacacactaatgggaacacctatttagaatggtacctgcagaaaccaggccagtctccaaagctcctgatctacaaagtttccaaccgattttctggggtcccagacaggttcagtggcagtggatctgggacagatttcatactcaagatcagcagagtggaggctgaggatctgggagtttattactgctttcaaggttcacatgttcctccgacgttcggtggaggcaccaagctggaagtcaaacgggctgatgctgcaccaactgtatccatcttcccaccatccagtgagcagttaacatctggaggtgcctctgttgtgtgcctgctgaataacttctatcctcgagaggccaaagtacagtggaaggtggataacgccctccaatcgggtaactcccaggagagtgtcacagagcaggacagcaaggacagcacctacagcctcagcagcaccctgacgctgagcaaagcagactacgagaaacacaaagtctacgcctgcgaagtcacccatcagggcctgagctcgcccgtcacaaagagcttcaacaggggagagtgttag

SEQ ID NO: 76 - protein, 457 aa, Artificial Sequence
  Comment
MKCSWIIFFLMAVVTGVNSEVQLQQSGSELVKSGASVKLSCTVSGFNFTDYYIHWVRQRTEQGLEWIGRIDPENDETTYAPKFQGKATMTADTSSNTAYLQLTSLTSEDTAVYYCARSTVLDYWGHGTTLTVSSKTTPPSVYPLAPGSAAQTNSMVTLGCLVKGYFPEPVTVTWNSGSLSSGVHTFPAVLQSDLYTLSSSVTVPSSTWPSETVTCNVAHPASSTKVDKKIVPRDCGCKPCICTVPEVSSVFIFPPKPKDVLTITLTPKVTCVVVDISKDDPEVQFSWFVDDVEVHTAQTQPREEQFNSTFRSVSELPIMHQDWLNGKEFKCRVNSAAFPAPIEKTISKTKGRPKAPQVYTIPPPKEQMAKDKVSLTCMITDFFPEDITVEWQWNGQPAENYKNTQPIMDTDGSYFVYSKLNVQKSNWEAGNTFTCSVLHEGLHNHHTEKSLSHSPGK

SEQ ID NO: 77 - protein, 468 aa, Artificial Sequence
  Comment
MKCSWIIFFLMAVVTGVNSEVQLQQSGSELVKSGASVKLSCTVSGFNFTDYYIHWVRQRTEQGLEWIGRIDPENDETTYAPKFQGKATMTADTSSNTAYLQLTSLTSEDTAVYYCARSTVLDYWGHGTTLTVSSASPTSSTKGPSVFPLAPSSKSTSGGTAALGCLVKDYFPEPVTVSWNSGALTSGVHTFPAVLQSSGLYSLSSVVTVPSSSLGTQTYICNVNHKPSNTKVDKKVEPKSCDKTHTCPPCPAPELLGGPSVFLFPPKPKDTLMISRTPEVTCVVVDVSHEDPEVKFNWYVDGVEVHNAKTKPREEQYNSTYRVVSVLTVLHQDWLNGKEYKCKVSNKALPAPIEKTISKAKGQPREPQVYTLPPSRDELTKNQVSLTCLVKGFYPSDIAVEWESNGQPENNYKTTPPVLDSDGSFFLYSKLTVDKSRWQQGNVFSCSVMHEGLHNHYTQKSLSLSPGK

SEQ ID NO: 78 - protein, 240 aa, Artificial Sequence
  Comment
MDMKLPVRLLVLMFWIPGFSSDVLMTQTPLSLPVSLGDQASISCRASQSIVHTNGNTYLEWYLQKPGQSPKLLIYKVSNRFSGVPDRFSGSGSGTDFILKISRVEAEDLGVYYCFQGSHVPPTFGGGTKLEVKRADAAPTVSIFPPSSEQLTSGGASVVCLLNNFYPREAKVQWKVDNALQSGNSQESVTEQDSKDSTYSLSSTLTLSKADYEKHKVYACEVTHQGLSSPVTKSFNRGEC

SEQ ID NO: 79 - protein, 5 aa, Artificial Sequence
  Artificial sequence
  misc_feature (1)..(1): Xaa represents a neutral and polar amino acid or a acidic polar amino acid
XYYIH

SEQ ID NO: 80 - protein, 16 aa, Artificial Sequence
  Artificial sequence
  misc_feature (7)..(7): Xaa represents a neutral and polar amino acid or a acidic polar amino acid
  misc_feature (8)..(8): Xaa represents a neutral and polar amino acid or a acidic polar amino acid
RIDPENXXTTYAPKFQ

SEQ ID NO: 81 - protein, 11 aa, Artificial Sequence
  Artificial sequence
  misc_feature (2)..(2): Xaa represents a non-polar amino acid or a neutral polar amino acid
RXSQSIVHTNG

SEQ ID NO: 82 - protein, 13 aa, Artificial Sequence
  Artificial sequence
  misc_feature (5)..(5): Xaa represents a non-polar amino acid
  misc_feature (13)..(13): Xaa represents a non-polar amino acid
SPASXSVSLGDRX